European Patent Application EP 4 371 976 A1, published May 22, 2024. Title: Ionizable lipids and lipid nanoparticles containing thereof. Applicant: CERTEST BIOTEC, S.L. The sequence listing filed with the application follows.

SEQUENCE LISTING (1 sequence)

SEQ ID NO: 1 - RNA, 2088 nt, synthetic construct
  source 1..2088: mol_type = other RNA
aggaggcacagacaccaaggacagagacgctggctaggccgccctccccactgttaccaacgccaccatggaggacgccaagaacatcaagaagggccccgcccccttctaccccctggaggacggcaccgccggcgagcagctgcacaaggccatgaagaggtacgccctggtgcccggcaccatcgccttcaccgacgcccacatcgaggtggacatcacctacgccgagtacttcgagatgagcgtgaggctggccgaggccatgaagaggtacggcctgaacaccaaccacaggatcgtggtgtgcagcgagaacagcctgcagttcttcatgcccgtgctgggcgccctgttcatcggcgtggccgtggcccccgccaacgacatctacaacgagagggagctgctgaacagcatgggcatcagccagcccaccgtggtgttcgtgagcaagaagggcctgcagaagatcctgaacgtgcagaagaagctgcccatcatccagaagatcatcatcatggacagcaagaccgactaccagggcttccagagcatgtacaccttcgtgaccagccacctgccccccggcttcaacgagtacgacttcgtgcccgagagcttcgacagggacaagaccatcgccctgatcatgaacagcagcggcagcaccggcctgcccaagggcgtggccctgccccacaggaccgcctgcgtgaggttcagccacgccagggaccccatcttcggcaaccagatcatccccgacaccgccatcctgagcgtggtgcccttccaccacggcttcggcatgttcaccaccctgggctacctgatctgcggcttcagggtggtgctgatgtacaggttcgaggaggagctgttcctgaggagcctgcaggactacaagatccagagcgccctgctggtgcccaccctgttcagcttcttcgccaagagcaccctgatcgacaagtacgacctgagcaacctgcacgagatcgccagcggcggcgcccccctgagcaaggaggtgggcgaggccgtggccaagaggttccacctgcccggcatcaggcagggctacggcctgaccgagaccaccagcgccatcctgatcacccccgagggcgacgacaagcccggcgccgtgggcaaggtggtgcccttcttcgaggccaaggtggtggacctggacaccggcaagaccctgggcgtgaaccagaggggcgagctgtgcgtgaggggccccatgatcatgagcggctacgtgaacaaccccgaggccaccaacgccctgatcgacaaggacggctggctgcacagcggcgacatcgcctactgggacgaggacgagcacttcttcatcgtggacaggctgaagagtctgatcaagtacaagggctaccaggtggcccccgccgagctggagagcatcctgctgcagcaccccaacatcttcgacgccggcgtggccggcctgcccgacgacgacgccggcgagctgcccgccgccgtggtggtgctggagcacggcaagaccatgaccgagaaggagatcgtggactacgtggccagccaggtgaccaccgccaagaagctgaggggcggcgtggtgttcgtggacgaggtgcccaagggcctgaccggcaagctggacgccaggaagatcagggagatcctgatcaaggccaagaagggcggcaagatcgccgtgtgatgagctcgctttcttgctgtccaatttctattaaaggttcctttgttccctaagtccaactactaaactgggggatattatgaagggccttgagcatctggattctgcctaataaaaaacatttattttcattgcgctcgctttcttgctgtccaatttctattaaaggttcctttgttccctaagtccaactactaaactgggggatattatgaagggccttgagcatctggattctgcctaataaaaaacatttattttcattgcaaaaaaaaaaaaaaaaaaaaaaaaaaaaaagaaaaaaaaaaaaaaaaaaaaaaaaaaaaaaaaaaaaaaaaaaaaaaaaaaaaaaaaaaaaaaaaaaaaaa